European Patent Specification EP 4 021 901 B1, published September 24, 2025. Title: SUBSTITUTED PYRIDOPYRIMIDINONYL COMPOUNDS USEFUL AS T CELL ACTIVATORS. Applicant: Bristol-Myers Squibb Company. The sequence listing filed with the application follows.

SEQUENCE LISTING (4 sequences)

SEQ ID NO: 1 - DNA, 2256 bp, Homo sapiens
atggccaaggagaggggcctaataagccccagtgattttgcccagctgcaaaaatacatggaatactccaccaaaaaggtcagtgatgtcctaaagctcttcgaggatggcgagatggctaaatatgtccaaggagatgccattgggtacgagggattccagcaattcctgaaaatctatctcgaagtggataatgttcccagacacctaagcctggcactgtttcaatcctttgagactggtcactgcttaaatgagacaaatgtgacaaaagatgtggtgtgtctcaatgatgtttcctgctacttttcccttctggagggtggtcggccagaagacaagttagaattcaccttcaagctgtacgacacggacagaaatgggatcctggacagctcagaagtggacaaaattatcctacagatgatgcgagtggctgaatacctggattgggatgtgtctgagctgaggccgattcttcaggagatgatgaaagagattgactatgatggcagtggctctgtctctcaagctgagtgggtccgggctggggccaccaccgtgccactgctagtgctgctgggtctggagatgactctgaaggacgacggacagcacatgtggaggcccaagaggttccccagaccagtctactgcaatctgtgcgagtcaagcattggtcttggcaaacagggactgagctgtaacctctgtaagtacactgttcacgaccagtgtgccatgaaagccctgccttgtgaagtcagcacctatgccaagtctcggaaggacattggtgtccaatcacatgtgtgggtgcgaggaggctgtgagtccgggcgctgcgaccgctgtcagaaaaagatccggatctaccacagtctgaccgggctgcattgtgtatggtgccacctagagatccacgatgactgcctgcaagcggtgggccatgagtgtgactgtgggctgctccgggatcacatcctgcctccatcttccatctatcccagtgtcctggcctctggaccggatcgtaaaaatagcaaaacaagccagaagaccatggatgatttaaatttgagcacctctgaggctctgcggattgaccctgttcctaacacccacccacttctcgtctttgtcaatcctaagagtggcgggaagcaggggcagagggtgctctggaagttccagtatatattaaaccctcgacaggtgttcaacctcctaaaggatggtcctgagatagggctccgattattcaaggatgttcctgatagccggattttggtgtgtggtggagacggcacagtaggctggattctagagaccattgacaaagctaacttgccagttttgcctcctgttgctgtgttgcccctgggtactggaaatgatctggctcgatgcctaagatggggaggaggttatgaaggacagaatctggcaaagatcctcaaggatttagagatgagtaaagtggtacatatggatcgatggtctgtggaggtgatacctcaacaaactgaagaaaaaagtgacccagtcccctttcaaatcatcaataactacttctctattggcgtggatgcctctattgctcatcgattccacatcatgcgagagaaatatccggagaagttcaacagcagaatgaagaacaagctatggtacttcgaatttgccacatctgaatccatcttctcaacatgcaaaaagctggaggagtctttgacagttgagatctgtgggaaaccgctggatctgagcaacctgtccctagaaggcatcgcagtgctaaacatccctagcatgcatggtggctccaacctctggggtgataccaggagaccccatggggatatctatgggatcaaccaggccttaggtgctacagctaaagtcatcaccgaccctgatatcctgaaaacctgtgtaccagacctaagtgacaagagactggaagtggttgggctggagggtgcaattgagatgggccaaatctataccaagctcaagaatgctggacgtcggctggccaagtgctctgagatcaccttccacaccacaaaaacccttcccatgcaaattgacggagaaccctggatgcagacgccctgtacaatcaagatcacccacaagaaccagatgcccatgctcatgggcccacccccccgctccaccaatttctttggcttcttgagcggatcctcggagacagtgcggtttcagggacaccaccaccatcaccactga

SEQ ID NO: 2 - protein, 737 aa, Homo sapiens
MASPSDFAQLQKYMEYSTKKVSDVLKLFEDGEMAKYVQGDAIGYEGFQQFLKIYLEVDNVPRHLSLALFQSFETGHCLNETNVTKDVVCLNDVSCYFSLLEGGRPEDKLEFTFKLYDTDRNGILDSSEVDKIILQMMRVAEYLDWDVSELRPILQEMMKEIDYDGSGSVSQAEWVRAGATTVPLLVLLGLEMTLKDDGQHMWRPKRFPRPVYCNLCESSIGLGKQGLSCNLCKYTVHDQCAMKALPCEVSTYAKSRKDIGVQSHVWVRGGCESGRCDRCQKKIRIYHSLTGLHCVWCHLEIHDDCLQAVGHECDCGLLRDHILPPSSIYPSVLASGPDRKNSKTSQKTMDDLNLSTSEALRIDPVPNTHPLLVFVNPKSGGKQGQRVLWKFQYILNPRQVFNLLKDGPEIGLRLFKDVPDSRILVCGGDGTVGWILETIDKANLPVLPPVAVLPLGTGNDLARCLRWGGGYEGQNLAKILKDLEMSKVVHMDRWSVEVIPQQTEEKSDPVPFQIINNYFSIGVDASIAHRFHIMREKYPEKFNSRMKNKLWYFEFATSESIFSTCKKLEESLTVEICGKPLDLSNLSLEGIAVLNIPSMHGGSNLWGDTRRPHGDIYGINQALGATAKVITDPDILKTCVPDLSDKRLEVVGLEGAIEMGQIYTKLKNAGRRLAKCSEITFHTTKTLPMQIDGEPWMQTPCTIKITHKNQMPMLMGPPPRSGSSETVRFQGHHHHHH

SEQ ID NO: 3 - protein, 2838 aa, Homo sapiens
ATGGAGCCGCGGGACGGTAGCCCCGAGGCCCGGAGCAGCGACTCCGAGTCGGCTTCCGCCTCGTCCAGCGGCTCCGAGCGCGACGCCGGTCCCGAGCCGGACAAGGCGCCGCGGCGACTCAACAAGCGGCGCTTCCCGGGGCTGCGGCTCTTCGGGCACAGGAAAGCCATCACGAAGTCGGGCCTCCAGCACCTGGCCCCCCCTCCGCCCACCCCTGGGGCCCCGTGCAGCGAGTCAGAGCGGCAGATCCGGAGTACAGTGGACTGGAGCGAGTCAGCGACATATGGGGAGCACATCTGGTTCGAGACCAACGTGTCCGGGGACTTCTGCTACGTTGGGGAGCAGTACTGTGTAGCCAGGATGCTGCAGAAGTCAGTGTCTCGAAGAAAGTGCGCAGCCTGCAAGATTGTGGTGCACACGCCCTGCATCGAGCAGCTGGAGAAGATAAATTTCCGCTGTAAGCCGTCCTTCCGTGAATCAGGCTCCAGGAATGTCCGCGAGCCAACCTTTGTACGGCACCACTGGGTACACAGACGACGCCAGGACGGCAAGTGTCGGCACTGTGGGAAGGGATTCCAGCAGAAGTTCACCTTCCACAGCAAGGAGATTGTGGCCATCAGCTGCTCGTGGTGCAAGCAGGCATACCACAGCAAGGTGTCCTGCTTCATGCTGCAGCAGATCGAGGAGCCGTGCTCGCTGGGGGTCCACGCAGCCGTGGTCATCCCGCCCACCTGGATCCTCCGCGCCCGGAGGCCCCAGAATACTCTGAAAGCAAGCAAGAAGAAGAAGAGGGCATCCTTCAAGAGGAAGTCCAGCAAGAAAGGGCCTGAGGAGGGCCGCTGGAGACCCTTCATCATCAGGCCCACCCCCTCCCCGCTCATGAAGCCCCTGCTGGTGTTTGTGAACCCCAAGAGTGGGGGCAACCAGGGTGCAAAGATCATCCAGTCTTTCCTCTGGTATCTCAATCCCCGACAAGTCTTCGACCTGAGCCAGGGAGGGCCCAAGGAGGCGCTGGAGATGTACCGCAAAGTGCACAACCTGCGGATCCTGGCGTGCGGGGGCGACGGCACGGTGGGCTGGATCCTCTCCACCCTGGACCAGCTACGCCTGAAGCCGCCACCCCCTGTTGCCATCCTGCCCCTGGGTACTGGCAACGACTTGGCCCGAACCCTCAACTGGGGTGGGGGCTACACAGATGAGCCTGTGTCCAAGATCCTCTCCCACGTGGAGGAGGGGAACGTGGTACAGCTGGACCGCTGGGACCTCCACGCTGAGCCCAACCCCGAGGCAGGGCCTGAGGACCGAGATGAAGGCGCCACCGACCGGTTGCCCCTGGATGTCTTCAACAACTACTTCAGCCTGGGCTTTGACGCCCACGTCACCCTGGAGTTCCACGAGTCTCGAGAGGCCAACCCAGAGAAATTCAACAGCCGCTTTCGGAATAAGATGTTCTACGCCGGGACAGCTTTCTCTGACTTCCTGATGGGCAGCTCCAAGGACCTGGCCAAGCACATCCGAGTGGTGTGTGATGGAATGGACTTGACTCCCAAGATCCAGGACCTGAAACCCCAGTGTGTTGTTTTCCTGAACATCCCCAGGTACTGTGCGGGCACCATGCCCTGGGGCCACCCTGGGGAGCACCACGACTTTGAGCCCCAGCGGCATGACGACGGCTACCTCGAGGTCATTGGCTTCACCATGACGTCGTTGGCCGCGCTGCAGGTGGGCGGACACGGCGAGCGGCTGACGCAGTGTCGCGAGGTGGTGCTCACCACATCCAAGGCCATCCCGGTGCAGGTGGATGGCGAGCCCTGCAAGCTTGCAGCCTCACGCATCCGCATCGCCCTGCGCAACCAGGCCACCATGGTGCAGAAGGCCAAGCGGCGGAGCGCCGCCCCCCTGCACAGCGACCAGCAGCCGGTGCCAGAGCAGTTGCGCATCCAGGTGAGTCGCGTCAGCATGCACGACTATGAGGCCCTGCACTACGACAAGGAGCAGCTCAAGGAGGCCTCTGTGCCGCTGGGCACTGTGGTGGTCCCAGGAGACAGTGACCTAGAGCTCTGCCGTGCCCACATTGAGAGACTCCAGCAGGAGCCCGATGGTGCTGGAGCCAAGTCCCCGACATGCCAGAAACTGTCCCCCAAGTGGTGCTTCCTGGACGCCACCACTGCCAGCCGCTTCTACAGGATCGACCGAGCCCAGGAGCACCTCAACTATGTGACTGAGATCGCACAGGATGAGATTTATATCCTGGACCCTGAGCTGCTGGGGGCATCGGCCCGGCCTGACCTCCCAACCCCCACTTCCCCTCTCCCCACCTCACCCTGCTCACCCACGCCCCGGTCACTGCAAGGGGATGCTGCACCCCCTCAAGGTGAAGAGCTGATTGAGGCTGCCAAGAGGAACGACTTCTGTAAGCTCCAGGAGCTGCACCGAGCTGGGGGCGACCTCATGCACCGAGACGAGCAGAGTCGCACGCTCCTGCACCACGCAGTCAGCACTGGCAGCAAGGATGTGGTCCGCTACCTGCTGGACCACGCCCCCCCAGAGATCCTTGATGCGGTGGAGGAAAACGGGGAGACCTGTTTGCACCAAGCAGCGGCCCTGGGCCAGCGCACCATCTGCCACTACATCGTGGAGGCCGGGGCCTCGCTCATGAAGACAGACCAGCAGGGCGACACTCCCCGGCAGCGGGCTGAGAAGGCTCAGGACACCGAGCTGGCCGCCTACCTGGAGAACCGGCAGCACTACCAGATGATCCAGCGGGAGGACCAGGAGACGGCTGTGGGATCCTCGGAGACAGTGCGGTTTCAGGGACACCACCACCATCACCACTGA

SEQ ID NO: 4 - protein, 945 aa, Homo sapiens
MEPRDGSPEARSSDSESASASSSGSERDAGPEPDKAPRRLNKRRFPGLRLFGHRKAITKSGLQHLAPPPPTPGAPCSESERQIRSTVDWSESATYGEHIWFETNVSGDFCYVGEQYCVARMLQKSVSRRKCAACKIVVHTPCIEQLEKINFRCKPSFRESGSRNVREPTFVRHHWVHRRRQDGKCRHCGKGFQQKFTFHSKEIVAISCSWCKQAYHSKVSCFMLQQIEEPCSLGVHAAVVIPPTWILRARRPQNTLKASKKKKRASFKRKSSKKGPEEGRWRPFIIRPTPSPLMKPLLVFVNPKSGGNQGAKIIQSFLWYLNPRQVFDLSQGGPKEALEMYRKVHNLRILACGGDGTVGWILSTLDQLRLKPPPPVAILPLGTGNDLARTLNWGGGYTDEPVSKILSHVEEGNVVQLDRWDLHAEPNPEAGPEDRDEGATDRLPLDVFNNYFSLGFDAHVTLEFHESREANPEKFNSRFRNKMFYAGTAFSDFLMGSSKDLAKHIRVVCDGMDLTPKIQDLKPQCVVFLNIPRYCAGTMPWGHPGEHHDFEPQRHDDGYLEVIGFTMTSLAALQVGGHGERLTQCREVVLTTSKAIPVQVDGEPCKLAASRIRIALRNQATMVQKAKRRSAAPLHSDQQPVPEQLRIQVSRVSMHDYEALHYDKEQLKEASVPLGTVVVPGDSDLELCRAHIERLQQEPDGAGAKSPTCQKLSPKWCFLDATTASRFYRIDRAQEHLNYVTEIAQDEIYILDPELLGASARPDLPTPTSPLPTSPCSPTPRSLQGDAAPPQGEELIEAAKRNDFCKLQELHRAGGDLMHRDEQSRTLLHHAVSTGSKDVVRYLLDHAPPEILDAVEENGETCLHQAAALGQRTICHYIVEAGASLMKTDQQGDTPRQRAEKAQDTELAAYLENRQHYQMIQREDQETAVGSSETVRFQGHHHHHH